European Patent Application EP 4 285 997 A1, published December 6, 2023. Title: Composition for improving joint function. Applicant: MEGMILK SNOW BRAND CO., LTD. The sequence listing filed with the application follows.

SEQUENCE LISTING (10 sequences)

SEQ ID NO: 1 - DNA, 19 bp, Artificial Sequence
  primer
gaggccaagccctggtatg

SEQ ID NO: 2 - DNA, 19 bp, Artificial Sequence
  primer
cgggccgattgatctcagc

SEQ ID NO: 3 - DNA, 19 bp, Artificial Sequence
  primer
ctgggctacactgagcacc

SEQ ID NO: 4 - DNA, 21 bp, Artificial Sequence
  primer
aagtggtcgttgagggcaatg

SEQ ID NO: 5 - DNA, 23 bp, Artificial Sequence
  primer
tcctgatgtgggtgaatacaatg

SEQ ID NO: 6 - DNA, 23 bp, Artificial Sequence
  primer
gccatcgtgaagtctggtaaaat

SEQ ID NO: 7 - DNA, 23 bp, Artificial Sequence
  primer
atgctgactatggctacaaaagc

SEQ ID NO: 8 - DNA, 19 bp, Artificial Sequence
  primer
tcgggcaatcatcaggcac

SEQ ID NO: 9 - DNA, 20 bp, Artificial Sequence
  primer
ggcagacccgcaacattact

SEQ ID NO: 10 - DNA, 19 bp, Artificial Sequence
  primer
caccaccgacctcgaagtc